European Patent Application EP 4 414 447 A1, published August 14, 2024. Title: MICROORGANISM HAVING ABILITY TO PRODUCE N- ACETYLNEURAMINIC ACID AND/OR N-ACETYLNEURAMINIC ACID-CONTAINING CARBOHYDRATE AND METHOD FOR PRODUCING N-ACETYLNEURAMINIC ACID AND/OR N-ACETYLNEURAMINIC ACID-CONTAINING CARBOHYDRATE USING SAID MICROORGANISM. Applicant: KYOWA HAKKO BIO CO., LTD. Application EP 22 878 639.8, filed October 7, 2022. The sequence listing filed with the application follows.

SEQUENCE LISTING (58 sequences)

SEQ ID NO: 1 - DNA, 1104 bp, Escherichia coli
  source 1..1104: mol_type = genomic DNA
gtgaatttactgacagtgagtactgatctcatcagtatttttttattcacgacactgtttctgttttttgcccgtaaggtggcaaaaaaagtcggtttagtggataaaccaaacttccgcaaacgtcaccaggggttgataccactcgttgggggtatttcggtttacgcagggatttgcttcacgttcggaattgtcgattactatattccgcatgcatctctctatctcgcttgtgccggtgtgcttgttttcattggcgcgctggatgaccgttttgatatcagcgtaaaaatccgtgccaccatacaggccgctgttggcattgttatgatggtgtttggcaacctttatctcagtagcctgggttatatctttggcttctgggagatggtgctcggaccgtttggttacttcctgacgctatttgccgtctgggcggccattaatgccttcaacatggttgatggcattgatggcttgctgggcgggttgtcctgcgtctcgtttgcagcaatcggtatgattttgtggttcgacgggcaaaccagcctcgcaatctggtgctttgcgatgatcgccgccatcctgccatatatcatgcttaaccttggtatcctgggtcgccgctacaaagtctttatgggtgatgcgggcagtacgctgattggttttaccgttatctggatcctgctcgaaacgacccagggcaaaacccatcccatcagcccggttaccgctttgtggataatcgccattccgctaatggatatggtggcgattatgtaccgtcgcctgcgtaaaggcatgagcccattctctcctgaccgtcagcatattcaccatttgatcatgcgtgccgggtttacttcccgtcaggcgtttgtgctgattaccattgccgcagcactgctcgcttccattggcgtgctggcagaatattctcattttgtcccggagtgggtcatgctggtgctctttttgctagcattcttcctctatggatattgcattaagcgtgcctggaaagttgctcgctttattaagcgcgtaaaacgcagactgcgtagaaatcgtggtggcagccccaatttaaccaaataa

SEQ ID NO: 2 - protein, 367 aa, Escherichia coli
MNLLTVSTDLISIFLFTTLFLFFARKVAKKVGLVDKPNFRKRHQGLIPLVGGISVYAGICFTFGIVDYYIPHASLYLACAGVLVFIGALDDRFDISVKIRATIQAAVGIVMMVFGNLYLSSLGYIFGFWEMVLGPFGYFLTLFAVWAAINAFNMVDGIDGLLGGLSCVSFAAIGMILWFDGQTSLAIWCFAMIAAILPYIMLNLGILGRRYKVFMGDAGSTLIGFTVIWILLETTQGKTHPISPVTALWIIAIPLMDMVAIMYRRLRKGMSPFSPDRQHIHHLIMRAGFTSRQAFVLITIAAALLASIGVLAEYSHFVPEWVMLVLFLLAFFLYGYCIKRAWKVARFIKRVKRRLRRNRGGSPNLTK

SEQ ID NO: 3 - DNA, 1131 bp, Escherichia coli
  source 1..1131: mol_type = genomic DNA
gtgaaagtactgactgtatttggtacgcgcccggaagccatcaagatggcgccgttggtgcatgcgttggcaaaagatcctttttttgaggctaaagtttgcgtcactgcgcagcatcgggagatgctcgatcaggtgctgaaactcttttccattgtacctgactacgatctcaacataatgcagccaggacagggcctgacagagataacctgtcggattctggaagggctaaaacctattcttgccgagttcaaaccagacgtcgtgctggttcacggcgacacaacgacgacgctggcaaccagcctggcggcgttttatcagcgtattcctgttggtcacgttgaggctggtctgcgcacgggcgatctctattcgccgtggccggaagaggctaaccgtacattgaccgggcatctggcgatgtatcacttctctccaaccgaaacttcccggcaaaacttgctgcgtgaaaacgttgcggatagccgaatcttcattaccggtaatacagttattgatgcactgttatgggtgcgtgaccaggtgatgagcagcgatacgctgcgttcagaactggcggcaaattacccgtttatcgaccccgataaaaagatgattctggtgaccggtcacaggcgtgagagcttcggtcgtggctttgaagaaatctgccatgcgctggcagacatcgccaccacgcaccaggacatccagattgtctatccggtgcatctcaacccgaacgtcagggagccggtcaatcgcattctggggcatgtgaaaaatgtcattctgatcgatcctcaggagtatttaccgtttgtctggctgatgaaccacgcctggctgattttgaccgactcaggcggcattcaggaagaagcgccttcgctggggaaaccggtgctggtgatgcgtgataccactgagcgtccggaagcggtgacggcgggtacggtgcgtctggtaggcacggataagcagcgaattgtcgaggaagtgacgcgtcttttaaaagacgaaaacgaatatcaagctatgagccgcgcccataacccgtatggtgatggtcaggcatgctctcgcattctggaagcgttaaaaaataatcggatatcactatga

SEQ ID NO: 4 - protein, 376 aa, Escherichia coli
MKVLTVFGTRPEAIKMAPLVHALAKDPFFEAKVCVTAQHREMLDQVLKLFSIVPDYDLNIMQPGQGLTEITCRILEGLKPILAEFKPDVVLVHGDTTTTLATSLAAFYQRIPVGHVEAGLRTGDLYSPWPEEANRTLTGHLAMYHFSPTETSRQNLLRENVADSRIFITGNTVIDALLWVRDQVMSSDTLRSELAANYPFIDPDKKMILVTGHRRESFGRGFEEICHALADIATTHQDIQIVYPVHLNPNVREPVNRILGHVKNVILIDPQEYLPFVWLMNHAWLILTDSGGIQEEAPSLGKPVLVMRDTTERPEAVTAGTVRLVGTDKQRIVEEVTRLLKDENEYQAMSRAHNPYGDGQACSRILEALKNNRISL

SEQ ID NO: 5 - DNA, 1263 bp, Escherichia coli
  source 1..1263: mol_type = genomic DNA
atgagttttgcgaccatttctgttatcggactgggttatatcgggctgccaacggcggcagcgtttgcctcacggcaaaaacaggtaattggtgtcgatatcaaccaacacgcggttgataccatcaatcgtggcgaaatccatatcgtcgaacctgatttggcgagtgtagtaaaaactgccgtagaaggtggttttttacgagcgagcacgacgccagttgaagcggatgcctggctgattgctgtacccacgccgtttaaaggcgatcatgagccagatatgacctacgttgaatcggctgctcgctccattgcgccagtgctgaaaaaaggcgcgctggtgatccttgaatccacctcgccggtggggtcaaccgagaagatggcagaatggttagcagagatgcgtccggatctcactttcccacagcaggtgggcgagcaggcggacgtcaacattgcttactgcccggaacgcgtgttaccgggccaggttatggtcgagctgattaaaaacgatcgcgtgattggtggtatgacgccggtttgttcggcccgcgccagcgaactgtacaaaattttcctcgaaggtgagtgtgtcgtcactaactcgcggacggcggaaatgtgtaagctcaccgaaaacagcttccgcgatgtgaatatcgcttttgctaatgaattgtcgctgatttgtgccgatcaggggattaacgtctgggaactgattcgcctggcgaatcgtcaccctcgcgttaatattcttcagcctggccctggcgtgggcggtcactgcattgctgttgatccgtggtttatcgtggcacagaacccccagcaggcgcggcttatccgtaccgcgcgcgaagtgaacgatcacaaaccgttctgggttatcgatcaggtgaaagcggcggtggctgattgcctggcggctaccgataaacgcgccagtgaactgaaaatcgcctgctttggtctggcgtttaaaccgaatattgatgacctgcgcgaaagcccggcgatggaaatcgctgaactgatcgcccagtggcatagcggcgaaactctggttgttgagcctaacatccaccagttgccgaaaaaactgaccgggctttgtactctggcgcagcttgacgaggcgctggcaacggcagacgtgctggtgatgctggtcgatcatagtcagttcaaagttatcaatggcgacaatgtccatcagcagtatgtcgtcgatgccaaaggagtctggcgctga

SEQ ID NO: 6 - protein, 420 aa, Escherichia coli
MSFATISVIGLGYIGLPTAAAFASRQKQVIGVDINQHAVDTINRGEIHIVEPDLASVVKTAVEGGFLRASTTPVEADAWLIAVPTPFKGDHEPDMTYVESAARSIAPVLKKGALVILESTSPVGSTEKMAEWLAEMRPDLTFPQQVGEQADVNIAYCPERVLPGQVMVELIKNDRVIGGMTPVCSARASELYKIFLEGECVVTNSRTAEMCKLTENSFRDVNIAFANELSLICADQGINVWELIRLANRHPRVNILQPGPGVGGHCIAVDPWFIVAQNPQQARLIRTAREVNDHKPFWVIDQVKAAVADCLAATDKRASELKIACFGLAFKPNIDDLRESPAMEIAELIAQWHSGETLVVEPNIHQLPKKLTGLCTLAQLDEALATADVLVMLVDHSQFKVINGDNVHQQYVVDAKGVWR

SEQ ID NO: 7 - DNA, 1041 bp, Campylobacter jejuni
  source 1..1041: mol_type = genomic DNA
atgaaagaaataaaaatacaaaatataatcataagtgaagaaaaagcacccttagtcgtgcctgaaataggcattaatcataatggcagtttagaactagctaaaattatggtagatgcagcctttagcgcaggtgctaagattataaagcatcaaacccacatcgttgaagatgagatgagtaaggccgctaaaaaagtaattcctggtaatgcaaaaataagcatttatgagattatgcaaaaatgtgctttagattataaagatgagctagcacttaaagaatacacagaaaaattaggtcttgtttatcttagcacacctttttctcgtgcaggtgcaaaccgcttagaagatatgggagttagtgcttttaagattggttcaggtgagtgtaataattatccgcttattaaacacatagcagcctttaaaaagcctatgatagttagcacaggaatgaatagtattgaaagtataaaaccaactgtaaaaatcttattagacaatgaaattccctttgttttaatgcacacgaccaatctttacccaaccccacataatcttgtaagattaaacgctatgcttgaattaaaaaaagaattttcttgcatggtaggcttaagcgaccacacaacagataatcttgcgtgtttaggtgcggttgcacttggtgcttgtgtgcttgaaagacattttactgatagtatggatagaagtggccctgatatagtttgttctatggatacaaaggctttaaaagagctaattatgcaaagtgagcaaatggctataatgagaggaaataatgaaagcaaaaaagcagctaagcaagaacaagttacaattgattttgcctttgcaagcgtagttagtattaaagatattaaaaaaggcgaagttttatctatggacaatatctgggttaaaagacctggacttggtggaattagtgcggttgaatttgaaaatattttaggcaaaaaagcattaagagatatagaaaatgatactcagttaagctatgaggattttgcgtga

SEQ ID NO: 8 - DNA, 1176 bp, Synechocystis sp. PCC6803
  source 1..1176: mol_type = genomic DNA
atgattgcccatcgccgtcaggagttagcccagcaatattaccaggctttacaccaggacgtattgcccttttgggaaaaatattccctcgatcgccaggggggcggttactttacctgcttagaccgtaaaggccaggtttttgacacagataaattcatttggttacaaaaccgtcaggtatggcagtttgccgttttctacaaccgtttggaaccaaaaccccaatggttagaaattgcccgccatggtgctgattttttagctcgccacggccgagatcaagacggtaattggtattttgctttggatcaggaaggcaaacccctgcgtcaaccctataacgttttttccgattgcttcgccgccatggcctttagtcaatatgccttagccagtggggcgcaggaagctaaagccattgccctgcaggcctacaataacgtcctacgccgtcagcacaatcccaaaggtcaatacgagaagtcctatccaggtactagacccctcaaatccctggcggtgccgatgattttagccaacctcaccctggagatggaatggttattaccgcctactaccgtggaagaggtgttggcccaaaccgtcagagaagtgatgacggatttcctcgacccagaaataggattaatgcgggaagcggtgacccccacaggagaatttgttgatagttttgaagggcggttgctcaacccaggacacggcattgaagccatgtggttcatgatggacattgcccaacgctccggcgatcgccagttacaggagcaagccattgcagtggtgttgaacaccctggaatatgcctgggatgaagaatttggtggcatattttatttccttgatcgccagggccaccctccccaacaactggaatgggaccaaaagctctggtgggtacatttggaaaccctggttgccctagccaagggccaccaagccactggccaagaaaaatgttggcaatggtttgagcgggtccatgattacgcctggagtcatttcgccgatcctgagtatggggaatggtttggctacctgaatcgccggggagaggtgttactcaacctaaaaggggggaaatggaaagggtgcttccacgtgccccgagctctgtggctctgtgcggaaactctccaacttccggttagttaa

SEQ ID NO: 9 - DNA, 480 bp, Saccharomyces cerevisiae S288C
  source 1..480: mol_type = genomic DNA
atgagcttacccgatggattttatataaggcgaatggaagagggggatttggaacaggtcactgagacgctaaaggttttgaccaccgtgggcactattacccccgaatccttcagcaaactcataaaatactggaatgaagccacagtatggaatgataacgaagataaaaaaataatgcaatataaccccatggtgattgtggacaagcgcaccgagacggttgccgctacggggaatatcatcatcgaaagaaagatcattcatgaactggggctatgtggccacatcgaggacattgcagtaaactccaagtatcagggccaaggtttgggcaagctcttgattcatcaattggtaactatcggctttgactacggttgttataagattattttagattgcgatgagaaaaatgtcaaattctatgaaaaatgtgggtttagcaacgcaggcgtggaaatgcaaattagaaaatag

SEQ ID NO: 10 - DNA, 34 bp, synthetic construct
  misc_feature 1..34: note = Description of the artificial sequence: base sequence of primerFw for amplification of CjneuB fragment
  source 1..34: mol_type = other DNA
cacaggaaacagaccatgaaagaaataaaaatac

SEQ ID NO: 11 - DNA, 20 bp, synthetic construct
  misc_feature 1..20: note = Description of the artificial sequence: base sequence of primerRv for amplification of CjneuB fragment
  source 1..20: mol_type = other DNA
tcacgcaaaatcctcatagc

SEQ ID NO: 12 - DNA, 35 bp, synthetic construct
  misc_feature 1..35: note = Description of the artificial sequence: base sequence of primerFw for amplification of slr1975 fragment
  source 1..35: mol_type = other DNA
gaggattttgcgtgaatgattgcccatcgccgtca

SEQ ID NO: 13 - DNA, 19 bp, synthetic construct
  misc_feature 1..19: note = Description of the artificial sequence: base sequence of primerRv for amplification of slr1975 fragment
  source 1..19: mol_type = other DNA
ttaactaaccggaagttgg

SEQ ID NO: 14 - DNA, 32 bp, synthetic construct
  misc_feature 1..32: note = Description of the artificial sequence: base sequence of primerFw for amplification of GNA1 fragment
  source 1..32: mol_type = other DNA
cttccggttagttaaatgagcttacccgatgg

SEQ ID NO: 15 - DNA, 36 bp, synthetic construct
  misc_feature 1..36: note = Description of the artificial sequence: base sequence of primerRv for amplification of GNA1 fragment
  source 1..36: mol_type = other DNA
ggatccccgggtaccctattttctaatttgcatttc

SEQ ID NO: 16 - DNA, 855 bp, Escherichia coli
  source 1..855: mol_type = genomic DNA
atggtactgatgatcgtcagcggacgttcaggttcaggtaaatctgtcgccctgcgtgcgctggaagatatgggtttttactgcgtggataaccttcccgtagtgttgttacccgatctggctcgaaccctggccgatcgcgagatttctgccgccgtcagcattgatgttcgtaatatgccggagtcaccagaaatattcgaacaggcgatgagtaacctgcctgacgctttctcaccgcaactcctgttcctggatgccgaccgtaataccttaattcgtcgttacagtgacacgcgccgactgcatccgctttccagcaaaaacctgtcgctggaaagtgctatcgacaaagaaagcgatttgctggagcctctgcgttcgcgagcggatctgattgtcgatacctcagaaatgtccgttcacgagctggctgaaatgctgcgtacccgtctgctgggtaaacgtgaacgcgaactgaccatggtctttgagtctttcggcttcaaacacggtatccctatcgatgcagattacgtctttgacgtgcgcttcttgccgaacccgcactgggatccgaaactgcgtccaatgacaggtcttgataaacctgtcgccgcgttcctcgaccgccacacagaagtacacaattttatctaccagacgcgaagctatcttgagctatggttacctatgctggaaaccaacaaccgtagctacttgacggtcgccattggttgtaccggcgggaagcaccgttcggtgtatattgcagagcaactggcagactacttccgctcgcgcggtaaaaacgtccagtcacgccatcgtacgctggaaaaacgtaaaccatga

SEQ ID NO: 17 - DNA, 20 bp, synthetic construct
  misc_feature 1..20: note = Description of the artificial sequence: base sequence of primerFw for cat fragment amplification
  source 1..20: mol_type = other DNA
accaggcgtttaagggcacc

SEQ ID NO: 18 - DNA, 45 bp, synthetic construct
  misc_feature 1..45: note = Description of the artificial sequence: base sequence of primerRv for cat fragment amplification
  source 1..45: mol_type = other DNA
gactacgggcctaaagtcgacagaataaataaatcctggtgtccc

SEQ ID NO: 19 - DNA, 28 bp, synthetic construct
  misc_feature 1..28: note = Description of the artificial sequence: base sequence of primerFw for sacB fragment amplification
  source 1..28: mol_type = other DNA
gtcgactttaggcccgtagtctgcaaat

SEQ ID NO: 20 - DNA, 21 bp, synthetic construct
  misc_feature 1..21: note = Description of the artificial sequence: base sequence of primerRv for sacB fragment amplification
  source 1..21: mol_type = other DNA
tacggttagccatttgcctgc

SEQ ID NO: 21 - DNA, 20 bp, synthetic construct
  misc_feature 1..20: note = Description of the artificial sequence: base sequence ofprimer_Fw for amplification of wecA upstream 1 fragment
  source 1..20: mol_type = other DNA
taccccaagtttaagaactc

SEQ ID NO: 22 - DNA, 37 bp, synthetic construct
  misc_feature 1..37: note = Description of the artificial sequence: base sequence ofprimer_Rv for amplification of wecA upstream 1 fragment
  source 1..37: mol_type = other DNA
gcctgaataagtgcggccgcaatgcatgctctcagag

SEQ ID NO: 23 - DNA, 38 bp, synthetic construct
  misc_feature 1..38: note = Description of the artificial sequence: base sequence ofprimer_Fw for amplification of wecA downstream 1 fragment
  source 1..38: mol_type = other DNA
aaatgccgatatgcggccgcatgaggatgtgatgacac

SEQ ID NO: 24 - DNA, 19 bp, synthetic construct
  misc_feature 1..19: note = Description of the artificial sequence: base sequence ofprimer_Rv for amplification of wecA downstream 1 fragment
  source 1..19: mol_type = other DNA
acaggttatctctgtcagg

SEQ ID NO: 25 - DNA, 20 bp, synthetic construct
  misc_feature 1..20: note = Description of the artificial sequence: base sequence ofprimer_Fw for amplification of wecA upstream 2 fragment
  source 1..20: mol_type = other DNA
taccccaagtttaagaactc

SEQ ID NO: 26 - DNA, 35 bp, synthetic construct
  misc_feature 1..35: note = Description of the artificial sequence: base sequence ofprimer_Rv for amplification of wecA upstream 2 fragment
  source 1..35: mol_type = other DNA
gtgtcatcacatcctcataatgcatgctctcagag

SEQ ID NO: 27 - DNA, 35 bp, synthetic construct
  misc_feature 1..35: note = Description of the artificial sequence: base sequence ofprimer_Fw for amplification of wecA downstream 2 fragment
  source 1..35: mol_type = other DNA
ctctgagagcatgcattatgaggatgtgatgacac

SEQ ID NO: 28 - DNA, 19 bp, synthetic construct
  misc_feature 1..19: note = Description of the artificial sequence: base sequence ofprimer_Rv for amplification of wecA downstream 2 fragment
  source 1..19: mol_type = other DNA
acaggttatctctgtcagg

SEQ ID NO: 29 - DNA, 20 bp, synthetic construct
  misc_feature 1..20: note = Description of the artificial sequence: base sequence ofprimer_Fw for making fragments for wecA destruction
  source 1..20: mol_type = other DNA
acctggctcgcatgcgtaag

SEQ ID NO: 30 - DNA, 18 bp, synthetic construct
  misc_feature 1..18: note = Description of the artificial sequence: base sequence ofprimer_Rv for making fragments for wecA destruction
  source 1..18: mol_type = other DNA
agtgacgcaaactttagc

SEQ ID NO: 31 - DNA, 19 bp, synthetic construct
  misc_feature 1..19: note = Description of the artificial sequence: base sequence ofprimer_Fw for amplification of wecB upstream 1 fragment
  source 1..19: mol_type = other DNA
atggtggcgattatgtacc

SEQ ID NO: 32 - DNA, 41 bp, synthetic construct
  misc_feature 1..41: note = Description of the artificial sequence: base sequence ofprimer_Rv for amplification of wecB upstream 1 fragment
  source 1..41: mol_type = other DNA
gcctgaataagtgcggccgcatcgattctcttcgaataagc

SEQ ID NO: 33 - DNA, 38 bp, synthetic construct
  misc_feature 1..38: note = Description of the artificial sequence: base sequence ofprimer_Fw for amplification of wecB downstream 1 fragment
  source 1..38: mol_type = other DNA
aaatgccgatatgcggccgcgttttgcgaccatttctg

SEQ ID NO: 34 - DNA, 20 bp, synthetic construct
  misc_feature 1..20: note = Description of the artificial sequence: base sequence ofprimer_Rv for amplification of wecB downstream 1 fragment
  source 1..20: mol_type = other DNA
caactttctcaaaggcaaag

SEQ ID NO: 35 - DNA, 19 bp, synthetic construct
  misc_feature 1..19: note = Description of the artificial sequence: base sequence ofprimer_Fw for amplification of wecB upstream 2 fragment
  source 1..19: mol_type = other DNA
atggtggcgattatgtacc

SEQ ID NO: 36 - DNA, 39 bp, synthetic construct
  misc_feature 1..39: note = Description of the artificial sequence: base sequence ofprimer_Rv for amplification of wecB upstream 2 fragment
  source 1..39: mol_type = other DNA
cagaaatggtcgcaaaacatcgattctcttcgaataagc

SEQ ID NO: 37 - DNA, 39 bp, synthetic construct
  misc_feature 1..39: note = Description of the artificial sequence: base sequence ofprimer_Fw for amplification of wecB downstream 2 fragment
  source 1..39: mol_type = other DNA
gcttattcgaagagaatcgatgttttgcgaccatttctg

SEQ ID NO: 38 - DNA, 20 bp, synthetic construct
  misc_feature 1..20: note = Description of the artificial sequence: base sequence ofprimer_Rv for amplification of wecB downstream 2 fragment
  source 1..20: mol_type = other DNA
caactttctcaaaggcaaag

SEQ ID NO: 39 - DNA, 20 bp, synthetic construct
  misc_feature 1..20: note = Description of the artificial sequence: base sequence ofprimer_Fw for making fragments for wecB destruction
  source 1..20: mol_type = other DNA
aggcgtttgtgctgattacc

SEQ ID NO: 40 - DNA, 20 bp, synthetic construct
  misc_feature 1..20: note = Description of the artificial sequence: base sequence ofprimer_Rv for making fragments for wecB destruction
  source 1..20: mol_type = other DNA
ttggcatcgacgacatactg

SEQ ID NO: 41 - DNA, 19 bp, synthetic construct
  misc_feature 1..19: note = Description of the artificial sequence: base sequence ofprimer_Fw for amplification of wecC upstream 1 fragment
  source 1..19: mol_type = other DNA
acctgattcagaaatgttc

SEQ ID NO: 42 - DNA, 39 bp, synthetic construct
  misc_feature 1..39: note = Description of the artificial sequence: base sequence ofprimer_Rv for amplification of wecC upstream 1 fragment
  source 1..39: mol_type = other DNA
gcctgaataagtgcggccgcatccgattattttttaacg

SEQ ID NO: 43 - DNA, 39 bp, synthetic construct
  misc_feature 1..39: note = Description of the artificial sequence: base sequence ofprimer_Fw for amplification of wecC downstream 1 fragment
  source 1..39: mol_type = other DNA
aaatgccgatatgcggccgctgagaaagattctgataac

SEQ ID NO: 44 - DNA, 19 bp, synthetic construct
  misc_feature 1..19: note = Description of the artificial sequence: base sequence ofprimer_Rv for amplification of wecC downstream 1 fragment
  source 1..19: mol_type = other DNA
acctgatagccaaaaatcg

SEQ ID NO: 45 - DNA, 19 bp, synthetic construct
  misc_feature 1..19: note = Description of the artificial sequence: base sequence ofprimer_Fw for amplification of wecC upstream 2 fragment
  source 1..19: mol_type = other DNA
acctgattcagaaatgttc

SEQ ID NO: 46 - DNA, 38 bp, synthetic construct
  misc_feature 1..38: note = Description of the artificial sequence: base sequence ofprimer_Rv for amplification of wecC upstream 2 fragment
  source 1..38: mol_type = other DNA
gttatcagaatctttctcaatccgattattttttaacg

SEQ ID NO: 47 - DNA, 38 bp, synthetic construct
  misc_feature 1..38: note = Description of the artificial sequence: base sequence ofprimer_Fw for amplification of wecC downstream 2 fragment
  source 1..38: mol_type = other DNA
cgttaaaaaataatcggattgagaaagattctgataac

SEQ ID NO: 48 - DNA, 19 bp, synthetic construct
  misc_feature 1..19: note = Description of the artificial sequence: base sequence ofprimer_Rv for amplification of wecC downstream 2 fragment
  source 1..19: mol_type = other DNA
acctgatagccaaaaatcg

SEQ ID NO: 49 - DNA, 20 bp, synthetic construct
  misc_feature 1..20: note = Description of the artificial sequence: base sequence ofprimer_Fw for making fragments for wecC destruction
  source 1..20: mol_type = other DNA
tcagacctatcgctatttgc

SEQ ID NO: 50 - DNA, 18 bp, synthetic construct
  misc_feature 1..18: note = Description of the artificial sequence: base sequence ofprimer_Rv for making fragments for wecC destruction
  source 1..18: mol_type = other DNA
tttcaccgatgataaagg

SEQ ID NO: 51 - DNA, 546 bp, Escherichia coli
  source 1..546: mol_type = genomic DNA
gtgcaggccaaaattgcggcatcaaatacgggtgaactggatgccctgcaacagctgggattctccctggtagaaggtgaagttgatttggcgctacccgtgaacaatgccagtgatagcggtgctgtagtggcacaagagaccgatattcccgcattacgtcagttagccagcgccgcatttgcgcaaagccgttttcgtgcgccgtggtatgcgcctgacgccagcagtcgcttttatgcacagtggattgaaaatgccgtgcgcggcacctttgatcatcaatgtctgattttacgtgcggcgtccggcgatattcgcggctatgtctctttacgggaactcaatgcgacagatgcgcgaattggcctgctggctggacgcggtgcaggtgctgagctgatgcaaacggcgctaaactgggcgtatgctcgcggtaaaacaactttgcgggtggcgacccaaatgggcaacaccgccgcgcttaaacgatacatacaaagtggtgcgaatgtagaaagcaccgcgtactggttatacaggtga

SEQ ID NO: 52 - protein, 181 aa, Escherichia coli
MQAKIAASNTGELDALQQLGFSLVEGEVDLALPVNNASDSGAVVAQETDIPALRQLASAAFAQSRFRAPWYAPDASSRFYAQWIENAVRGTFDHQCLILRAASGDIRGYVSLRELNATDARIGLLAGRGAGAELMQTALNWAYARGKTTLRVATQMGNTAALKRYIQSGANVESTAYWLYR

SEQ ID NO: 53 - DNA, 1131 bp, Escherichia coli
  source 1..1131: mol_type = genomic DNA
atgattccatttaacgcaccgccggtggtgggaaccgaactcgactatatgcagtcggcaatgggtagcggcaaactgtgtggcgatggcggttttacccgtcgctgccagcagtggctggagcaacgttttggcagcgccaaagtgttactgacgccgtcctgcaccgcttcgctggagatggcggcgctgctgctcgatatccagcctggcgatgaagtgatcatgccgagctacacctttgtctccaccgccaatgcctttgtgctgcgtggcgcaaaaatcgtttttgtggatgttcgcccggacaccatgaacatcgacgaaacgctgattgaagcggcgatcaccgacaaaacgcgcgttatcgtgccggtccattacgcgggtgtggcctgcgaaatggacaccattatggcgttggcgaaaaagcataatctgtttgtggtagaagatgccgctcagggcgtgatgtccacttacaaagggcgtgcactgggaaccattggtcatattggctgctttagcttccatgaaaccaaaaactatacggcgggtggtgaaggcggcgcgacgctgattaacgataaagcgttaatcgaacgagccgagatcatccgtgaaaagggcactaaccgcagccagttcttccgtggtcaggtcgataaatatacctggcgcgatattggctccagctatttgatgtccgatctgcaagctgcgtacctgtgggcgcaactggaagcagcggatcgtatcaaccagcaacgtctggcgctgtggcaaaactactacgatgcgttagcgcctctggcgaaagccgggcgtatcgagctgccgtcgattcccgatggctgcgtgcagaacgcgcatatgttctacattaaactgcgggatattgatgaccggagcgcgttgattaactttctgaaagaagcggaaatcatggcggtgttccattacattccgctgcacggttgccctgcgggggaacgctttggtgagttccacggtgaagatcgctacaccaccaaagagagcgagcgcctgctgcgcctgccgctgttctacaacctgtcgcccgtcaatcagcgtacggtaattgcgactttgttgaactacttctcctga

SEQ ID NO: 54 - protein, 376 aa, Escherichia coli
MIPFNAPPVVGTELDYMQSAMGSGKLCGDGGFTRRCQQWLEQRFGSAKVLLTPSCTASLEMAALLLDIQPGDEVIMPSYTFVSTANAFVLRGAKIVFVDVRPDTMNIDETLIEAAITDKTRVIVPVHYAGVACEMDTIMALAKKHNLFVVEDAAQGVMSTYKGRALGTIGHIGCFSFHETKNYTAGGEGGATLINDKALIERAEIIREKGTNRSQFFRGQVDKYTWRDIGSSYLMSDLQAAYLWAQLEAADRINQQRLALWQNYYDALAPLAKAGRIELPSIPDGCVQNAHMFYIKLRDIDDRSALINFLKEAEIMAVFHYIPLHGCPAGERFGEFHGEDRYTTKESERLLRLPLFYNLSPVNQRTVIATLLNYFS

SEQ ID NO: 55 - DNA, 1080 bp, Escherichia coli
  source 1..1080: mol_type = genomic DNA
atgactgtactgattcacgtactgggatcggatatccctcaccataaccgaaccgttttgcggtttttcaatgacgcgctggctgcgacgagcgagcacgcgcgcgagtttatggttgttggcaaggacgacggcttaagtgatagctgtccggcgctttctgtgcaatttttccctgggaaaaaatcgctggcggaagcggtcatcgcgaaagcaaaagctaaccgtcagcagcgttttttcttccacggtcagttcaatcccacactgtggctggctctgctgagtggtggcattaagcccagccagtttttctggcatatctggggggcagacctgtatgagctttccagtggcttgagatataagcttttttacccactacgtcgcctggcgcaaaagcgagtcggctgtgtatttgccacccgcggcgatttgagcttttttgccaaaacgcatccaaaggtgcggggcgaactgctgtacttcccgacgcggatggacccttctctcaatacgatggcgaacgatcggcaacgtgaagggaaaatgaccattctggtggggaactccggtgaccgcagcaatgaccatattgctgccttgtgcgccgttcatcagcaatttggcgatacggtaaaagtggtggtgccgatgggatatccgcctaataacgaagcgtacattgaggaagttcgtcaggcggggctggagttattcagcgaagaaaatctgcaaattttgagcgaaaaactggaatttgacgcctatctggcgctacttcgtcagtgcgatcttggttactttatttttgcccgccagcagggcattggtacgctttgcttactgattcaggcgggcattccttgtgtgcttaaccgggaaaatccgttctggcaggatatgacggaacagcatttgccggtgctgtttactaccgacgatctcaacgaggatattgtgcgtgaagcgcagcgccagttggcgtcggtggataaaaacaccattgccttctttagccctaactatctacaaggctggcagcgggcgttggcgattgccgccggggaggtcgcatga

SEQ ID NO: 56 - protein, 359 aa, Escherichia coli
MTVLIHVLGSDIPHHNRTVLRFFNDALAATSEHAREFMVVGKDDGLSDSCPALSVQFFPGKKSLAEAVIAKAKANRQQRFFFHGQFNPTLWLALLSGGIKPSQFFWHIWGADLYELSSGLRYKLFYPLRRLAQKRVGCVFATRGDLSFFAKTHPKVRGELLFFPTRMDPSLNTMANDRQREGKMTILVGNSGDRSNEHIAALRAVHQQFGDTVKVVVPMGYPPNNEAYIEEVRQAGLELFSEENLQILSEKLEFDAYLALLRQCDLGYFIFARQQGIGTLCLLIQAGIPCVLNRENPFWQDMTEQHLPVLFTTDDLNEDIVREAQRQLASVDKNTIAFFSPNYLQGWQRALAIAAREVA

SEQ ID NO: 57 - DNA, 741 bp, Escherichia coli
  source 1..741: mol_type = genomic DNA
atgaataacaacaccacggcaccaacctatacgctgcgtggcttacagttgattggttggcgtgatatgcagcacgccctcgattatctgtttgctgacgggcagcttaagcagggaacgctggttgccattaatgctgaaaaaatgctgactattgaagataacgccgaggtcagggagttaattaacgctgccgaatttaaatatgcggatggcatcagcgttgtacgttcagtacgtaaaaagtacccgcaggcgcaggtttcccgcgttgccggtgccgatctctgggaagagctgatggcgcgcgcaggcaaagaagggacgccggtatttcttgtgggcggtaaacctgaagtgctggcgcaaactgaagctaaactgcgcaaccagtggaatgtgaatatcgttggcagtcaggatggttattttaaacccgagcagcgtcaggcgctgtttgaacgcattcatgccagcggtgcgcaaatcgtcaccgttgcgatgggatcgccaaagcaggagatcatcatgcgcgactgccgtctggtacatccagatgcgctgtatatgggcgttggcgggacttacgatgttttcaccggtcacgtaaaacgcgcaccgaaaatctggcaaacgctggggctggagtggctctaccgcctgctttcgcagccgagccgcattaagcgtcagcttcgtttgctgcgttatttacgctggcactacaccggcaacctatga

SEQ ID NO: 58 - protein, 246 aa, Escherichia coli
MNNNTTAPTYTLRGLQLIGWRDMQHALDYLFADGQLKQGTLVAINAEKMLTIEDNAEVRELINAAEFKYADGISVVRSVRKKYPQAQVSRVAGADLWEELMARAGKEGTPVFLVGGKPEVLAQTEAKLRNQWNVNIVGSQDGYFKPEQRQALFERIHASGAQIVTVAMGSPKQEIIMRDCRLVHPDALYMGVGGTYDVFTGHVKRAPKIWQTLGLEWLYRLLSQPSRIKRQLRLLRYLRWHYTGNL